European Patent Application EP 4 502 148 A1, published February 5, 2025. Title: 一种通用型细胞及其制备方法. Applicant: 士泽生物医药（苏州）有限公司. The sequence listing filed with the application follows.

SEQUENCE LISTING (41 sequences)

SEQ ID NO: 1 - protein, 225 aa, synthetic construct
MGRAMVARLGLGLLLLALLLPTQIYSSETTTGTSSNSSQSTSNSGLAPNPTNATTKAAGGGGGSGGGGSGGGGSNILIVIFPIFAILLFWGQFGIKTLKYRSGGMDEKTIALLVAGLVITVIVIVGAILFVPGEYSLKNATGLGLIVTSTGILILLHYYVFSTAIGLTSFVIAILVIQVIAYILAVVGLSLCIAACIPMHGPLLISGLSILALAQLLGLVYMKFV

SEQ ID NO: 2 - DNA, 20 bp, synthetic construct
  source 1..20: mol_type = other DNA
cgtgagtaaacctgaatctt

SEQ ID NO: 3 - DNA, 20 bp, synthetic construct
  source 1..20: mol_type = other DNA
agtcacatggttcacacggc

SEQ ID NO: 4 - DNA, 20 bp, synthetic construct
  source 1..20: mol_type = other DNA
gatattggcataagcctccc

SEQ ID NO: 5 - DNA, 20 bp, synthetic construct
  source 1..20: mol_type = other DNA
catcgctgttaagaagctcc

SEQ ID NO: 6 - protein, 164 aa, Homo sapiens
NILIVIFPIFAILLFWGQFGIKTLKYRSGGMDEKTIALLVAGLVITVIVIVGAILFVPGEYSLKNATGLGLIVTSTGILILLHYYVFSTAIGLTSFVIAILVIQVIAYILAVVGLSLCIAACIPMHGPLLISGLSILALAQLLGLVYMKFVASNQKTIQPPRNN

SEQ ID NO: 7 - protein, 152 aa, Homo sapiens
NILIVIFPIFAILLFWGQFGIKTLKYRSGGMDEKTIALLVAGLVITVIVIVGAILFVPGEYSLKNATGLGLIVTSTGILILLHYYVFSTAIGLTSFVIAILVIQVIAYILAVVGLSLCIAACIPMHGPLLISGLSILALAQLLGLVYMKFVE

SEQ ID NO: 8 - protein, 151 aa, Homo sapiens
NILIVIFPIFAILLFWGQFGIKTLKYRSGGMDEKTIALLVAGLVITVIVIVGAILFVPGEYSLKNATGLGLIVTSTGILILLHYYVFSTAIGLTSFVIAILVIQVIAYILAVVGLSLCIAACIPMHGPLLISGLSILALAQLLGLVYMKFV

SEQ ID NO: 9 - protein, 171 aa, Homo sapiens
NILIVIFPIFAILLFWGQFGIKTLKYRSGGMDEKTIALLVAGLVITVIVIVGAILFVPGEYSLKNATGLGLIVTSTGILILLHYYVFSTAIGLTSFVIAILVIQVIAYILAVVGLSLCIAACIPMHGPLLISGLSILALAQLLGLVYMKFVASNQKTIQPPRKAVEEPLNE

SEQ ID NO: 10 - protein, 182 aa, Homo sapiens
NILIVIFPIFAILLFWGQFGIKTLKYRSGGMDEKTIALLVAGLVITVIVIVGAILFVPGEYSLKNATGLGLIVTSTGILILLHYYVFSTAIGLTSFVIAILVIQVIAYILAVVGLSLCIAACIPMHGPLLISGLSILALAQLLGLVYMKFVASNQKTIQPPRKAVEEPLNAFKESKGMMNDE

SEQ ID NO: 11 - protein, 26 aa, Homo sapiens
MGRAMVARLGLGLLLLALLLPTQIYS

SEQ ID NO: 12 - protein, 54 aa, Homo sapiens
SETTTGTSSNSSQSTSNSGLAPNPTNATTKAAGGALQSTASLFVVSLSLLHLYS

SEQ ID NO: 13 - protein, 59 aa, Homo sapiens
MGRAMVARLGLGLLLLALLLPTQIYSSETTTGTSSNSSQSTSNSGLAPNPTNATTKAAG

SEQ ID NO: 14 - protein, 50 aa, Homo sapiens
MGRAMVARLGLGLLLLALLLPTQIYSSETTTGTSSNSSQSTSNSGLAPNP

SEQ ID NO: 15 - protein, 30 aa, Homo sapiens
TNATTKAAGGALQSTASLFVVSLSLLHLYS

SEQ ID NO: 16 - protein, 24 aa, Homo sapiens
SETTTGTSSNSSQSTSNSGLAPNP

SEQ ID NO: 17 - DNA, 22 bp, synthetic construct
  source 1..22: mol_type = other DNA
tggggccaaatcatgtagactc

SEQ ID NO: 18 - DNA, 22 bp, synthetic construct
  source 1..22: mol_type = other DNA
tcagtgggggtgaattcagtgt

SEQ ID NO: 19 - DNA, 21 bp, synthetic construct
  source 1..21: mol_type = other DNA
cagaagtccttgagagcctcc

SEQ ID NO: 20 - DNA, 22 bp, synthetic construct
  source 1..22: mol_type = other DNA
tgtgcatcagtatctcagcagg

SEQ ID NO: 21 - DNA, 22 bp, synthetic construct
  source 1..22: mol_type = other DNA
ctgtgcctctaccacttctatg

SEQ ID NO: 22 - DNA, 22 bp, synthetic construct
  source 1..22: mol_type = other DNA
ccttccatgtcacacaacagcc

SEQ ID NO: 23 - DNA, 22 bp, synthetic construct
  source 1..22: mol_type = other DNA
tggaatccacactttccagttc

SEQ ID NO: 24 - DNA, 20 bp, synthetic construct
  source 1..20: mol_type = other DNA
tggagtctccgttcctccag

SEQ ID NO: 25 - DNA, 20 bp, synthetic construct
  source 1..20: mol_type = other DNA
aagatgagtatgcctgccgt

SEQ ID NO: 26 - DNA, 20 bp, synthetic construct
  source 1..20: mol_type = other DNA
atgcggcatcttcaaacctc

SEQ ID NO: 27 - DNA, 21 bp, synthetic construct
  source 1..21: mol_type = other DNA
cctggagcttcttaacagcga

SEQ ID NO: 28 - DNA, 21 bp, synthetic construct
  source 1..21: mol_type = other DNA
tgtgtcgggttctgagtagag

SEQ ID NO: 29 - protein, 305 aa, Homo sapiens
MWPLVAALLLGSACCGSAQLLFNKTKSVEFTFCNDTVVIPCFVTNMEAQNTTEVYVKWKFKGRDIYTFDGALNKSTVPTDFSSAKIEVSQLLKGDASLKMDKSDAVSHTGNYTCEVTELTREGETIIELKYRVVSWFSPNENILIVIFPIFAILLFWGQFGIKTLKYRSGGMDEKTIALLVAGLVITVIVIVGAILFVPGEYSLKNATGLGLIVTSTGILILLHYYVFSTAIGLTSFVIAILVIQVIAYILAVVGLSLCIAACIPMHGPLLISGLSILALAQLLGLVYMKFVASNQKTIQPPRNN

SEQ ID NO: 30 - DNA, 918 bp, Homo sapiens
  source 1..918: mol_type = genomic DNA
atgtggcccctggtagcggcgctgttgctgggctcggcgtgctgcggatcagctcagctactatttaataaaacaaaatctgtagaattcacgttttgtaatgacactgtcgtcattccatgctttgttactaatatggaggcacaaaacactactgaagtatacgtaaagtggaaatttaaaggaagagatatttacacctttgatggagctctaaacaagtccactgtccccactgactttagtagtgcaaaaattgaagtctcacaattactaaaaggagatgcctctttgaagatggataagagtgatgctgtctcacacacaggaaactacacttgtgaagtaacagaattaaccagagaaggtgaaacgatcatcgagctaaaatatcgtgttgtttcatggttttctccaaatgaaaatattcttattgttattttcccaatttttgctatactcctgttctggggacagtttggtattaaaacacttaaatatagatccggtggtatggatgagaaaacaattgctttacttgttgctggactagtgatcactgtcattgtcattgttggagccattcttttcgtcccaggtgaatattcattaaagaatgctactggccttggtttaattgtgacttctacagggatattaatattacttcactactatgtgtttagtacagcgattggattaacctccttcgtcattgccatattggttattcaggtgatagcctatatcctcgctgtggttggactgagtctctgtattgcggcgtgtataccaatgcatggccctcttctgatttcaggtttgagtatcttagctctagcacaattacttggactagtttatatgaaatttgtggcttccaatcagaagactatacaacctcctaggaataactga

SEQ ID NO: 31 - DNA, 20 bp, synthetic construct
  source 1..20: mol_type = other DNA
ccagatctacagcagcgaga

SEQ ID NO: 32 - DNA, 20 bp, synthetic construct
  source 1..20: mol_type = other DNA
gttcttcaggctgtactcgc

SEQ ID NO: 33 - DNA, 20 bp, synthetic construct
  source 1..20: mol_type = other DNA
gttcttcaggctgtactcgc

SEQ ID NO: 34 - DNA, 20 bp, synthetic construct
  source 1..20: mol_type = other DNA
ccaggatgtaggcgatcacc

SEQ ID NO: 35 - protein, 186 aa, synthetic construct
MWPLVAALLLGSACCGSAQLLFNKTKSVEFTFCNDTVVIPCFVTNMEAQNTTEVYVKWKFKGRDIYTFDGALNKSTVPTDFSSAKIEVSQLLKGDASLKMDKSDAVSHTGNYTCEVTELTREGETIIELKYRVVSWFSPNEGGGGSGGGGSGGGGSTNATTKAAGGALQSTASLFVVSLSLLHLYS

SEQ ID NO: 36 - protein, 233 aa, synthetic construct
MGRAMVARLGLGLLLLALLLPTQIYSSETTTGTSSNSSQSTSNSGLAPNPGGGGSGGGGSGGGGSQLLFNKTKSVEFTFCNDTVVIPCFVTNMEAQNTTEVYVKWKFKGRDIYTFDGALNKSTVPTDFSSAKIEVSQLLKGDASLKMDKSDAVSHTGNYTCEVTELTREGETIIELKYRVVSWFSPNEGGGGSGGGGSGGGGSTNATTKAAGGALQSTASLFVVSLSLLHLYS

SEQ ID NO: 37 - protein, 339 aa, synthetic construct
MGRAMVARLGLGLLLLALLLPTQIYSSETTTGTSSNSSQSTSNSGLAPNPGGGGSGGGGSGGGGSQLLFNKTKSVEFTFCNDTVVIPCFVTNMEAQNTTEVYVKWKFKGRDIYTFDGALNKSTVPTDFSSAKIEVSQLLKGDASLKMDKSDAVSHTGNYTCEVTELTREGETIIELKYRVVSWFSPNENILIVIFPIFAILLFWGQFGIKTLKYRSGGMDEKTIALLVAGLVITVIVIVGAILFVPGEYSLKNATGLGLIVTSTGILILLHYYVFSTAIGLTSFVIAILVIQVIAYILAVVGLSLCIAACIPMHGPLLISGLSILALAQLLGLVYMKFV

SEQ ID NO: 38 - protein, 210 aa, synthetic construct
MWPLVAALLLGSACCGSAQLLFNKTKSVEFTFCNDTVVIPCFVTNMEAQNTTEVYVKWKFKGRDIYTFDGALNKSTVPTDFSSAKIEVSQLLKGDASLKMDKSDAVSHTGNYTCEVTELTREGETIIELKYRVVSWFSPNEGGGGSGGGGSGGGGSSETTTGTSSNSSQSTSNSGLAPNPTNATTKAAGGALQSTASLFVVSLSLLHLYS

SEQ ID NO: 39 - protein, 347 aa, synthetic construct
MWPLVAALLLGSACCGSAQLLFNKTKSVEFTFCNDTVVIPCFVTNMEAQNTTEVYVKWKFKGRDIYTFDGALNKSTVPTDFSSAKIEVSQLLKGDASLKMDKSDAVSHTGNYTCEVTELTREGETIIELKYRVVSWFSPNEGGGGSGGGGSGGGGSSETTTGTSSNSSQSTSNSGLAPNPGGGGSGGGGSGGGGSSNILIVIFPIFAILLFWGQFGIKTLKYRSGGMDEKTIALLVAGLVITVIVIVGAILFVPGEYSLKNATGLGLIVTSTGILILLHYYVFSTAIGLTSFVIAILVIQVIAYILAVVGLSLCIAACIPMHGPLLISGLSILALAQLLGLVYMKFV

SEQ ID NO: 40 - protein, 293 aa, Homo sapiens
MWPLVAALLLGSACCGSAQLLFNKTKSVEFTFCNDTVVIPCFVTNMEAQNTTEVYVKWKFKGRDIYTFDGALNKSTVPTDFSSAKIEVSQLLKGDASLKMDKSDAVSHTGNYTCEVTELTREGETIIELKYRVVSWFSPNENILIVIFPIFAILLFWGQFGIKTLKYRSGGMDEKTIALLVAGLVITVIVIVGAILFVPGEYSLKNATGLGLIVTSTGILILLHYYVFSTAIGLTSFVIAILVIQVIAYILAVVGLSLCIAACIPMHGPLLISGLSILALAQLLGLVYMKFVE

SEQ ID NO: 41 - protein, 80 aa, Homo sapiens
MGRAMVARLGLGLLLLALLLPTQIYSSETTTGTSSNSSQSTSNSGLAPNPTNATTKAAGGALQSTASLFVVSLSLLHLYS